European Patent Specification EP 3 517 624 B1, published October 2, 2024. Title: System for predicting prognosis and benefit from adjuvant chemotherapy for patients with stage II and III gastric cancer. Applicant: Novomics Co., Ltd. The sequence listing filed with the application follows.

SEQUENCE LISTING (27 sequences)

SEQ ID NO: 1 - DNA, 22 bp, Artificial Sequence
  SFRP4 forward primer
ggagacttccgacttccttaca

SEQ ID NO: 2 - DNA, 20 bp, Artificial Sequence
  SFRP4 reverse primer
tggccttacataggctgtcc

SEQ ID NO: 3 - DNA, 20 bp, Artificial Sequence
  GZMB forward primer
cggtggcttcctgatacaag

SEQ ID NO: 4 - DNA, 20 bp, Artificial Sequence
  GZMB reverse primer
ttatggagcttccccaacag

SEQ ID NO: 5 - DNA, 20 bp, Artificial Sequence
  WARS forward primer
ttgtggacccatggacagta

SEQ ID NO: 6 - DNA, 20 bp, Artificial Sequence
  WARS reverse primer
ccaaaccgaacaatgagctt

SEQ ID NO: 7 - DNA, 20 bp, Artificial Sequence
  CDX1 forward primer
agggaggaacgtggtcaact

SEQ ID NO: 8 - DNA, 20 bp, Artificial Sequence
  CDX1 reverse primer
tatgatgggggcaggtagaa

SEQ ID NO: 9 - DNA, 20 bp, Artificial Sequence
  ACTB forward primer
tcaccctgaagtaccccatc

SEQ ID NO: 10 - DNA, 20 bp, Artificial Sequence
  ACTB reverse primer
tgtggtgccagattttctcc

SEQ ID NO: 11 - DNA, 20 bp, Artificial Sequence
  ATP5E forward primer
atggtggcctactggagaca

SEQ ID NO: 12 - DNA, 21 bp, Artificial Sequence
  ATP5E reverse primer
ctctcactgcttttgcacaga

SEQ ID NO: 13 - DNA, 21 bp, Artificial Sequence
  HPRT1 forward primer
tggtcaggcagtataatccaa

SEQ ID NO: 14 - DNA, 20 bp, Artificial Sequence
  HPRT1 reverse primer
cttcgtggggtccttttcac

SEQ ID NO: 15 - DNA, 18 bp, Artificial Sequence
  GPX1 forward primer
cccgtgcaaccagtttgg

SEQ ID NO: 16 - DNA, 23 bp, Artificial Sequence
  GPX1 reverse primer
ggacgtacttgagggaattcaga

SEQ ID NO: 17 - DNA, 20 bp, Artificial Sequence
  UBB forward primer
tgggtgagcttgtttgtgtc

SEQ ID NO: 18 - DNA, 21 bp, Artificial Sequence
  UBB reverse primer
tttgacctgttagcggatacc

SEQ ID NO: 19 - DNA, 20 bp, Artificial Sequence
  SFRP4 probe
aggcaatgcccagcctcatc

SEQ ID NO: 20 - DNA, 21 bp, Artificial Sequence
  GZMB probe
cgacttcgtgctgacagctgc

SEQ ID NO: 21 - DNA, 22 bp, Artificial Sequence
  WARS probe
tgccttttgcactgcttgtctg

SEQ ID NO: 22 - DNA, 20 bp, Artificial Sequence
  CDX1 probe
tgcctcttcctgcagcctca

SEQ ID NO: 23 - DNA, 20 bp, Artificial Sequence
  ACTB probe
cggcatcgtcaccaactggg

SEQ ID NO: 24 - DNA, 27 bp, Artificial Sequence
  ATP5E probe
tggactcagctacatccgatactccca

SEQ ID NO: 25 - DNA, 21 bp, Artificial Sequence
  HPRT1 probe
tgcaagcttgcgaccttgacc

SEQ ID NO: 26 - DNA, 27 bp, Artificial Sequence
  GPX1 probe
ctcttcgttcttggcgttctcctgatg

SEQ ID NO: 27 - DNA, 20 bp, Artificial Sequence
  UBB probe
caccaaccacgtccacccac